European Patent Application EP 4 588 938 A2, published July 23, 2025. Title: STABILIZED FORMULATIONS CONTAINING ANTI-INTERLEUKIN-6 RECEPTOR (IL-6R) ANTIBODIES. Applicant: REGENERON PHARMACEUTICALS, INC. Application EP, filed January 7, 2011. The sequence listing filed with the application follows.

SEQUENCE LISTING (74 sequences)

SEQ ID NO: 1 - DNA, 379 bp, synthetic construct
  misc_feature 1..379: note = Synthetic
  source 1..379: mol_type = other DNA
gaagtgcagctggtggagtctgggggaaacttggtacagcctggcaggtccctgagactctcctgtgcagcctctggattcatctttgatgattatgccatgcactgggtccggcaagctccagggaagggcctggagtgggtctcaggtattagttggaatagtggtagcataggctatgcggactctgtgaagggccgattcaccatctccagagacaacgccaagaactccctgtatctgcaaatgaacagtctgagagctgaggacacggccttgtattactgtgcaaaagatggaggcagcagctggttaccgttcgtctactactacggtatggacgtctggggccaagggaccacggtcaccgtctcgtcag

SEQ ID NO: 2 - protein, 126 aa, synthetic construct
  REGION 1..126: note = Synthetic
EVQLVESGGNLVQPGRSLRLSCAASGFIFDDYAMHWVRQAPGKGLEWVSGISWNSGSIGYADSVKGRFTISRDNAKNSLYLQMNSLRAEDTALYYCAKDGGSSWLPFVYYYGMDVWGQGTTVTVSS

SEQ ID NO: 3 - DNA, 24 bp, synthetic construct
  misc_feature 1..24: note = Synthetic
  source 1..24: mol_type = other DNA
ggattcatctttgatgattatgcc

SEQ ID NO: 4 - protein, 8 aa, synthetic construct
  REGION 1..8: note = Synthetic
GFIFDDYA

SEQ ID NO: 5 - DNA, 24 bp, synthetic construct
  misc_feature 1..24: note = Synthetic
  source 1..24: mol_type = other DNA
attagttggaatagtggtagcata

SEQ ID NO: 6 - protein, 8 aa, synthetic construct
  REGION 1..8: note = Synthetic
ISWNSGSI

SEQ ID NO: 7 - DNA, 57 bp, synthetic construct
  misc_feature 1..57: note = Synthetic
  source 1..57: mol_type = other DNA
gcaaaagatggaggcagcagctggttaccgttcgtctactactacggtatggacgtc

SEQ ID NO: 8 - protein, 19 aa, synthetic construct
  REGION 1..19: note = Synthetic
AKDGGSSWLPFVYYYGMDV

SEQ ID NO: 9 - DNA, 325 bp, synthetic construct
  misc_feature 1..325: note = Synthetic
  source 1..325: mol_type = other DNA
gaaatagtgatgacgcagtctccagccaccctgtctgtgtctcccggggaaagagccaccctctcctgcagggccagtcagagtattagcagcaactttgcctggtaccagcagaaacctggccaggctcccaggctcctcatctatggtgcatccaccagggccactggtatcccagccaggttcagtggcagtgggtctgggacagacttcactctcaccatcagcagcctgcagtctgaagattttgcagtttattactgtcagcagtatagtagctggcctccgtacacttttggccaggggaccaagctggagatcaaac

SEQ ID NO: 10 - protein, 108 aa, synthetic construct
  REGION 1..108: note = Synthetic
EIVMTQSPATLSVSPGERATLSCRASQSISSNFAWYQQKPGQAPRLLIYGASTRATGIPARFSGSGSGTDFTLTISSLQSEDFAVYYCQQYSSWPPYTFGQGTKLEIK

SEQ ID NO: 11 - DNA, 18 bp, synthetic construct
  misc_feature 1..18: note = Synthetic
  source 1..18: mol_type = other DNA
cagagtattagcagcaac

SEQ ID NO: 12 - protein, 6 aa, synthetic construct
  REGION 1..6: note = Synthetic
QSISSN

SEQ ID NO: 13-14 - skipped (2 entries)

SEQ ID NO: 15 - DNA, 30 bp, synthetic construct
  misc_feature 1..30: note = Synthetic
  source 1..30: mol_type = other DNA
cagcagtatagtagctggcctccgtacact

SEQ ID NO: 16 - protein, 10 aa, synthetic construct
  REGION 1..10: note = Synthetic
QQYSSWPPYT

SEQ ID NO: 17 - DNA, 349 bp, synthetic construct
  misc_feature 1..349: note = Synthetic
  source 1..349: mol_type = other DNA
gaagtgcagctggtggagtctgggggaggcttggttcagcctggcaggtccctgagactctcctgtgcagcctctagatttacctttgatgattatgccatgcactgggtccggcaagctccagggaagggcctggagtgggtctcaggtattagttggaatagtggtagaataggttatgcggactctgtgaagggccgattcaccatctccagagacaacgccgagaactccctctttctgcaaatgaacggtctgagagcagaggacacggccttgtattactgtgcaaaaggccgagattcttttgatatctggggccaagggacaatggtcaccgtctcttcag

SEQ ID NO: 18 - protein, 116 aa, synthetic construct
  REGION 1..116: note = Synthetic
EVQLVESGGGLVQPGRSLRLSCAASRFTFDDYAMHWVRQAPGKGLEWVSGISWNSGRIGYADSVKGRFTISRDNAENSLFLQMNGLRAEDTALYYCAKGRDSFDIWGQGTMVTVSS

SEQ ID NO: 19 - DNA, 24 bp, synthetic construct
  misc_feature 1..24: note = Synthetic
  source 1..24: mol_type = other DNA
agatttacctttgatgattatgcc

SEQ ID NO: 20 - protein, 8 aa, synthetic construct
  REGION 1..8: note = Synthetic
RFTFDDYA

SEQ ID NO: 21 - DNA, 24 bp, synthetic construct
  misc_feature 1..24: note = Synthetic
  source 1..24: mol_type = other DNA
attagttggaatagtggtagaata

SEQ ID NO: 22 - protein, 8 aa, synthetic construct
  REGION 1..8: note = Synthetic
ISWNSGRI

SEQ ID NO: 23 - DNA, 27 bp, synthetic construct
  misc_feature 1..27: note = Synthetic
  source 1..27: mol_type = other DNA
gcaaaaggccgagattcttttgatatc

SEQ ID NO: 24 - protein, 9 aa, synthetic construct
  REGION 1..9: note = Synthetic
AKGRDSFDI

SEQ ID NO: 25 - DNA, 322 bp, synthetic construct
  misc_feature 1..322: note = Synthetic
  source 1..322: mol_type = other DNA
gacatccagatgacccagtctccatcttccgtgtctgcatctgtaggagacagagtcaccatcacttgtcgggcgagtcagggtattagcagctggttagcctggtatcagcagaaaccagggaaagcccctaagctcctgatctatggtgcatccagtttggaaagtggggtcccatcaaggttcagcggcagtggatctgggacagatttcactctcaccatcagcagcctgcagcctgaagattttgcaagttattattgtcaacaggctaacagtttcccgtacacttttggccaggggaccaagctggagatcaaac

SEQ ID NO: 26 - protein, 107 aa, synthetic construct
  REGION 1..107: note = Synthetic
DIQMTQSPSSVSASVGDRVTITCRASQGISSWLAWYQQKPGKAPKLLIYGASSLESGVPSRFSGSGSGTDFTLTISSLQPEDFASYYCQQANSFPYTFGQGTKLEIK

SEQ ID NO: 27 - DNA, 18 bp, synthetic construct
  misc_feature 1..18: note = Synthetic
  source 1..18: mol_type = other DNA
cagggtattagcagctgg

SEQ ID NO: 28 - protein, 6 aa, synthetic construct
  REGION 1..6: note = Synthetic
QGISSW

SEQ ID NO: 29-30 - skipped (2 entries)

SEQ ID NO: 31 - DNA, 27 bp, synthetic construct
  misc_feature 1..27: note = Synthetic
  source 1..27: mol_type = other DNA
caacaggctaacagtttcccgtacact

SEQ ID NO: 32 - protein, 9 aa, synthetic construct
  REGION 1..9: note = Synthetic
QQANSFPYT

SEQ ID NO: 33 - DNA, 349 bp, synthetic construct
  misc_feature 1..349: note = Synthetic
  source 1..349: mol_type = other DNA
gaagtgcagctggtggagtctgggggaggcttggtacagcctggcaggtccctgagactctcctgtgcagcctctggattcacctttgatgattatgccctgcactgggtccggcaagctccagggaagggcctggagtgggtctcaggtgttagttggaatggtggtagaataggctatgcggactctgtgaaaggccgattcaccatctccagagacaacgccaagaactccctctttctgcaaatgaacagtctgagagttgaggacacggccttgtattattgtgcaaaaggccgggatgcttttgatatctggggccaagggacattggtcaccgtctcttcag

SEQ ID NO: 34 - protein, 116 aa, synthetic construct
  REGION 1..116: note = Synthetic
EVQLVESGGGLVQPGRSLRLSCAASGFTFDDYALHWVRQAPGKGLEWVSGVSWNGGRIGYADSVKGRFTISRDNAKNSLFLQMNSLRVEDTALYYCAKGRDAFDIWGQGTLVTVSS

SEQ ID NO: 35 - DNA, 24 bp, synthetic construct
  misc_feature 1..24: note = Synthetic
  source 1..24: mol_type = other DNA
ggattcacctttgatgattatgcc

SEQ ID NO: 36 - protein, 8 aa, synthetic construct
  REGION 1..8: note = Synthetic
GFTFDDYA

SEQ ID NO: 37 - DNA, 24 bp, synthetic construct
  misc_feature 1..24: note = Synthetic
  source 1..24: mol_type = other DNA
gttagttggaatggtggtagaata

SEQ ID NO: 38 - protein, 8 aa, synthetic construct
  REGION 1..8: note = Synthetic
VSWNGGRI

SEQ ID NO: 39 - DNA, 27 bp, synthetic construct
  misc_feature 1..27: note = Synthetic
  source 1..27: mol_type = other DNA
gcaaaaggccgggatgcttttgatatc

SEQ ID NO: 40 - protein, 9 aa, synthetic construct
  REGION 1..9: note = Synthetic
AKGRDAFDI

SEQ ID NO: 41 - DNA, 322 bp, synthetic construct
  misc_feature 1..322: note = Synthetic
  source 1..322: mol_type = other DNA
gacatccagatgacccagtctccatcttccgtgtctgcatctgtaggagacagagtcaccatcacttgtcgggcgagtcagggtattagcagctggttagcctggtatcagcagaaaccagggaaagcccctaaactcctgatctatgctgcatccagtttgcaaagtggggtcccatcaaggttcagcggcagtggatctgggacagatttcactctcaccatcagcagcctgcagcctgaagattttgcaacttactattgtcaacatgcttacagtttcccgtacacttttggccaggggaccaagctggagatcaaac

SEQ ID NO: 42 - protein, 107 aa, synthetic construct
  REGION 1..107: note = Synthetic
DIQMTQSPSSVSASVGDRVTITCRASQGISSWLAWYQQKPGKAPKLLIYAASSLQSGVPSRFSGSGSGTDFTLTISSLQPEDFATYYCQHAYSFPYTFGQGTKLEIK

SEQ ID NO: 43 - DNA, 18 bp, synthetic construct
  misc_feature 1..18: note = Synthetic
  source 1..18: mol_type = other DNA
cagggtattagcagctgg

SEQ ID NO: 44 - protein, 6 aa, synthetic construct
  REGION 1..6: note = Synthetic
QGISSW

SEQ ID NO: 45-46 - skipped (2 entries)

SEQ ID NO: 47 - DNA, 27 bp, synthetic construct
  misc_feature 1..27: note = Synthetic
  source 1..27: mol_type = other DNA
caacatgcttacagtttcccgtacact

SEQ ID NO: 48 - protein, 9 aa, synthetic construct
  REGION 1..9: note = Synthetic
QHAYSFPYT

SEQ ID NO: 49 - DNA, 361 bp, synthetic construct
  misc_feature 1..361: note = Synthetic
  source 1..361: mol_type = other DNA
caggtgcagctggtgcagtctggggctgaggtgaaagagcctggggcctcagtgaaggtctcctgcaaggcttctggatacaccttcacctcttatgatatcatctgggtgcgacaggccactggacaagggcttgagtggatgggatggatgaacccaaacagtggtaacacaggctatacacagaacctccagggcagagtcaccttgaccaggaacacctccataactacagtctacatggaactgagcagcctgagctctgaggacacggccgtttattactgtgcgcgagactacagtagccactactacggtttggacgtctggggccaagggaccacggtcaccgtctcctcaa

SEQ ID NO: 50 - protein, 120 aa, synthetic construct
  REGION 1..120: note = Synthetic
QVQLVQSGAEVKEPGASVKVSCKASGYTFTSYDIIWVRQATGQGLEWMGWMNPNSGNTGYTQNLQGRVTLTRNTSITTVYMELSSLSSEDTAVYYCARDYSSHYYGLDVWGQGTTVTVSS

SEQ ID NO: 51 - DNA, 24 bp, synthetic construct
  misc_feature 1..24: note = Synthetic
  source 1..24: mol_type = other DNA
ggatacaccttcacctcttatgat

SEQ ID NO: 52 - protein, 8 aa, synthetic construct
  REGION 1..8: note = Synthetic
GYTFTSYD

SEQ ID NO: 53 - DNA, 24 bp, synthetic construct
  misc_feature 1..24: note = Synthetic
  source 1..24: mol_type = other DNA
atgaacccaaacagtggtaacaca

SEQ ID NO: 54 - protein, 8 aa, synthetic construct
  REGION 1..8: note = Synthetic
MNPNSGNT

SEQ ID NO: 55 - DNA, 39 bp, synthetic construct
  misc_feature 1..39: note = Synthetic
  source 1..39: mol_type = other DNA
gcgcgagactacagtagccactactacggtttggacgtc

SEQ ID NO: 56 - protein, 13 aa, synthetic construct
  REGION 1..13: note = Synthetic
ARDYSSHYYGLDV

SEQ ID NO: 57 - DNA, 322 bp, synthetic construct
  misc_feature 1..322: note = Synthetic
  source 1..322: mol_type = other DNA
gacatccagttgacccagtctccatccttcctgtctacatctataggagacagagtcaccatcacttgctgggccagtcaggacattagcaattatttagcctggtatcagcaaaaaccagggaaagcccctaagctcctgatctttgttgcatccactttgcagagtggggtcccatcaaggttcagcggcagtggatctgggacagaattcactctcacaatcagtagcctgcagcctgaggattttgcaacttattactgtcaacagtttaatagttacccgctcactttcggcggagggaccaaggtggaaatcaaac

SEQ ID NO: 58 - protein, 107 aa, synthetic construct
  REGION 1..107: note = Synthetic
DIQLTQSPSFLSTSIGDRVTITCWASQDISNYLAWYQQKPGKAPKLLIFVASTLQSGVPSRFSGSGSGTEFTLTISSLQPEDFATYYCQQFNSYPLTFGGGTKVEIK

SEQ ID NO: 59 - DNA, 18 bp, synthetic construct
  misc_feature 1..18: note = Synthetic
  source 1..18: mol_type = other DNA
caggacattagcaattat

SEQ ID NO: 60 - protein, 6 aa, synthetic construct
  REGION 1..6: note = Synthetic
QDISNY

SEQ ID NO: 61-62 - skipped (2 entries)

SEQ ID NO: 63 - DNA, 30 bp, synthetic construct
  misc_feature 1..30: note = Synthetic
  source 1..30: mol_type = other DNA
caacagtttaatagttacccgctcactttc

SEQ ID NO: 64 - protein, 10 aa, synthetic construct
  REGION 1..10: note = Synthetic
QQFNSYPLTF

SEQ ID NO: 65-70 - skipped (6 entries)

SEQ ID NO: 71 - protein, 330 aa, synthetic construct [sequence omitted]

SEQ ID NO: 72 - protein, 327 aa, synthetic construct
  REGION 1..327: note = Synthetic
ASTKGPSVFPLAPCSRSTSESTAALGCLVKDYFPEPVTVSWNSGALTSGVHTFPAVLQSSGLYSLSSVVTVPSSSLGTKTYTCNVDHKPSNTKVDKRVESKYGPPCPSCPAPEFLGGPSVFLFPPKPKDTLMISRTPEVTCVVVDVSQEDPEVQFNWYVDGVEVHNAKTKPREEQFNSTYRVVSVLTVLHQDWLNGKEYKCKVSNKGLPSSIEKTISKAKGQPREPQVYTLPPSQEEMTKNQVSLTCLVKGFYPSDIAVEWESNGQPENNYKTTPPVLDSDGSFFLYSRLTVDKSRWQEGNVFSCSVMHEALHNHYTQKSLSLSLGK

SEQ ID NO: 73 - protein, 327 aa, synthetic construct
  REGION 1..327: note = Synthetic
ASTKGPSVFPLAPCSRSTSESTAALGCLVKDYFPEPVTVSWNSGALTSGVHTFPAVLQSSGLYSLSSVVTVPSSSLGTKTYTCNVDHKPSNTKVDKRVESKYGPPCPPCPAPEFLGGPSVFLFPPKPKDTLMISRTPEVTCVVVDVSQEDPEVQFNWYVDGVEVHNAKTKPREEQFNSTYRVVSVLTVLHQDWLNGKEYKCKVSNKGLPSSIEKTISKAKGQPREPQVYTLPPSQEEMTKNQVSLTCLVKGFYPSDIAVEWESNGQPENNYKTTPPVLDSDGSFFLYSRLTVDKSRWQEGNVFSCSVMHEALHNHYTQKSLSLSLGK

SEQ ID NO: 74 - protein, 358 aa, Homo sapiens
MVAVGCALLAALLAAPGAALAPRRCPAQEVARGVLTSLPGDSVTLTCPGVEPEDNATVHWVLRKPAAGSHPSRWAGMGRRLLLRSVQLHDSGNYSCYRAGRPAGTVHLLVDVPPEEPQLSCFRKSPLSNVVCEWGPRSTPSLTTKAVLLVRKFQNSPAEDFQEPCQYSQESQKFSCQLAVPEGDSSFYIVSMCVASSVGSKFSKTQTFQGCGILQPDPPANITVTAVARNPRWLSVTWQDPHSWNSSFYRLRFELRYRAERSKTFTTWMVKDLQHHCVIHDAWSGLRHVVQLRAQEEFGQGEWSEWSPEAMGTPWTESRSPPAENEVSTPMQALTTNKDDDNILFRDSANATSLPVQD